European Patent Application EP 4 130 277 A1, published February 8, 2023. Title: COLLAGENASE PREPARATION AND USE THEREOF. Applicant: AMANO ENZYME INC. The sequence listing filed with the application follows.

SEQUENCE LISTING (6 sequences)

SEQ ID NO: 1 - protein, 987 aa, Lysinibacillus fusiformis
DTQQLQEQYSMAELNNMSNRELIHTLGSIRWYQITDLFQFNDDTKAFYQNEERMQVIINELGNRGNSFTKEDSKGIETFVEVLRSAFYVAFYNNELGYLNERSFQDKCLPALNEIAKNPNFKLGTDEQDKVVSAYGKLIGNASSDVETVQHATNILKQYNENLSTYESENSKGQAIYDIIHGIDYDLQSYLYDTRKEANTTMWYGKIDSFIEEVNNIALIHNVTDSNSWLINNGIYYAGRLGQFHSNPNKGLEVVTQAMHMYPYLSEAYFVAVEQITTNYGGRDLNGNTVDLQKVREEGKKQYLPKTYTFDDGSIVFKTGDQVTEDKIQRLYWAAKEVKAQYHRVIGNDQALEPGNADDILTVVIYNSPDQYRLNRQLYGYETNNGGIYIEETGTFFTYERTPEQSIYSLEELFRHEYTHFLQGRFEVPGLFGTGDMYQNERLTWFQEGNAEFFAGSTRTNDVVPRKSIISGLSQDPSQRYTAEQTMFATYGSWDFYNYSFALQSYMYTHQFDMFDRIQDLIRANDVKNYDAYRDTLSKDSQLNMEYQAYMQQLIDNQETYEVPQVAEDYLMPHEPKALNEVQQEIVDIAHVKDANMTKHQSQFFNTFTLEGTYVGSATQGESQDWKTMSKQVNQMLEQLSQKEWSGYKTMTAYFVNYRVNAANQFEYDVVFHGVSTDDGETQAPIVQVNGPYTGMINEKIQFNSDGSKDTDGEIVSYLWDFGDGATSEAANPTHVYENEGTYKVTLTVKNNKGQESKGQTTATVQKGGQTGQEHAMIIPFNKPLKGSLIENDTNVYQFDITSPEEIDISVVNENQIGMTWVLYHESDKENYVAYGQEDGQTIKGKYNAKPGKYYLYVYKFDDEDGTYTVQVQNSTKTEIEPNNRPEEATMLPFHTPLSGSLMEDDHTDVYEFNVTSPKEIDISVLNENQIGMTWVLYHESDSQNYASFGQEDGNMINGKLNAKPGKYYLYVYKFENENGTYTVHVQ

SEQ ID NO: 2 - protein, 1072 aa, Lysinibacillus fusiformis
MKKKFTFNQLLIGVSTMAISLGGLQAEASAAEKTPYNVLQMKPIGIEMSKDEMVHSTMAEETLSYEERLEMGDFSQRPAPIMEQMDTQQLQEQYSMAELNNMSNRELIHTLGSIRWYQITDLFQFNDDTKAFYQNEERMQVIINELGNRGNSFTKEDSKGIETFVEVLRSAFYVAFYNNELGYLNERSFQDKCLPALNEIAKNPNFKLGTDEQDKVVSAYGKLIGNASSDVETVQHATNILKQYNENLSTYESENSKGQAIYDIIHGIDYDLQSYLYDTRKEANTTMWYGKIDSFIEEVNNIALIHNVTDSNSWLINNGIYYAGRLGQFHSNPNKGLEVVTQAMHMYPYLSEAYFVAVEQITTNYGGRDLNGNTVDLQKVREEGKKQYLPKTYTFDDGSIVFKTGDQVTEDKIQRLYWAAKEVKAQYHRVIGNDQALEPGNADDILTVVIYNSPDQYRLNRQLYGYETNNGGIYIEETGTFFTYERTPEQSIYSLEELFRHEYTHFLQGRFEVPGLFGTGDMYQNERLTWFQEGNAEFFAGSTRTNDVVPRKSIISGLSQDPSQRYTAEQTMFATYGSWDFYNYSFALQSYMYTHQFDMFDRIQDLIRANDVKNYDAYRDTLSKDSQLNMEYQAYMQQLIDNQETYEVPQVAEDYLMPHEPKALNEVQQEIVDIAHVKDANMTKHQSQFFNTFTLEGTYVGSATQGESQDWKTMSKQVNQMLEQLSQKEWSGYKTMTAYFVNYRVNAANQFEYDVVFHGVSTDDGETQAPIVQVNGPYTGMINEKIQFNSDGSKDTDGEIVSYLWDFGDGATSEAANPTHVYENEGTYKVTLTVKNNKGQESKGQTTATVQKGGQTGQEHAMIIPFNKPLKGSLIENDTNVYQFDITSPEEIDISVVNENQIGMTWVLYHESDKENYVAYGQEDGQTIKGKYNAKPGKYYLYVYKFDDEDGTYTVQVQNSTKTEIEPNNRPEEATMLPFHTPLSGSLMEDDHTDVYEFNVTSPKEIDISVLNENQIGMTWVLYHESDSQNYASFGQEDGNMINGKLNAKPGKYYLYVYKFENENGTYTVHVQ

SEQ ID NO: 3 - DNA, 2964 bp, Lysinibacillus fusiformis
gatacacagcaattgcaggagcagtactcgatggcagagcttaataatatgagcaatcgtgagcttatccatacgcttggcagtatccgttggtaccaaattacagacttattccaattcaatgatgacacaaaagctttttatcaaaatgaagagcgcatgcaagtaatcatcaatgaattagggaatagaggaaattcgtttacgaaggaagattcaaaggggatcgaaacatttgttgaggtattgcgttctgctttttatgtagcgttttataataatgaactaggctatttaaatgagagaagtttccaagataagtgtttaccagcattaaatgaaatagccaaaaatccaaactttaaacttggtacagatgagcaagataaagttgtatctgcctatggaaaattaataggtaatgcttctagtgatgtggaaaccgttcaacatgctacgaacattttaaaacaatataatgaaaatctttctacctatgaaagtgagaattcaaaaggacaagctatttacgatataatacacggcattgattatgatttgcagtcttatttatatgacactcgtaaagaggccaatacaacgatgtggtatgggaagattgatagcttcatagaggaagttaataacattgccctaatacataatgtgacggatagcaatagttggttaattaataatggcatttattatgcagggcgtttagggcagttccatagcaatcctaataagggtttagaagtcgttacacaagcgatgcatatgtatccctatttaagtgaagcttattttgtggcagtagagcaaattacgacaaattatggtggacgtgacttaaacggaaatacggttgatttacaaaaagtacgtgaagaaggaaaaaaacagtatctaccgaaaacatatacatttgatgatggatcaattgtattcaaaacgggagatcaagtaacggaagataaaattcaaagattatactgggctgcaaaagaggtaaaggcacaatatcatcgtgtaatcgggaatgatcaagcactagagcctggtaatgctgacgatatcttaaccgttgtcatttataactctcccgatcagtaccgattaaaccgacaattgtacggatatgaaacaaataatggtggtatttatattgaagagactggaacattctttacatatgaacgtacacctgagcaaagtatttatagcttagaagagctgttccgtcatgaatatacgcactttttacaaggtagatttgaggtgcctggtctattcgggacgggtgatatgtatcaaaatgagcgactaacatggttccaggaagggaatgcagaattttttgcagggtcaacacgtacaaatgacgttgtgcctcgtaagagcattattagtggattgtcacaggatccatcacaacgctatactgctgaacaaacaatgtttgccacatatggttcctgggatttttataattattcatttgcattacagtcttatatgtatacgcatcaattcgatatgtttgatagaattcaagatttaatccgcgcgaacgatgtgaaaaattatgatgcctatcgtgacactttaagtaaagattcacagctgaatatggaataccaagcatatatgcagcaattgatcgataaccaagaaacatacgaagtaccacaagtagcagaggattatttaatgccgcatgaaccaaaagcgttaaacgaagtacagcaagaaattgtcgatattgcacatgtgaaagatgcaaatatgacgaaacaccagtctcaattttttaatacgtttacactcgagggaacatatgtaggtagtgcaacacagggtgaatctcaagattggaaaacgatgagtaagcaagtaaaccaaatgctggagcaactgtctcaaaaagagtggagcggctataaaacaatgactgcgtactttgtcaactatcgtgtaaatgcggcaaaccagttcgagtatgatgtagtcttccatggcgtttccactgatgacggagaaacgcaagcaccaattgtacaagtaaatggtccatatactggcatgatcaatgaaaaaattcaatttaatagtgatgggtcaaaggatacggatggagaaatagtttcttatctttgggattttggtgatggcgcgacaagtgaagcagcaaatcctactcatgtatacgaaaatgaaggaacttacaaagtgacgttaaccgtgaaaaataataagggacaagaaagtaaagggcaaacaactgccactgtacagaaaggaggacagacagggcaagaacatgcgatgattattccatttaataaaccactaaaaggtagtttgatagaaaatgatacaaatgtctatcaatttgacattacatcgccagaagaaatagatatttctgtcgtaaatgaaaatcaaattggcatgacatgggtgctttatcatgaatctgataaggaaaactatgtagcgtatggacaggaagatggacagacaataaaaggtaagtacaatgcgaaaccaggaaagtattatttatacgtttataagtttgatgatgaagatggaacatataccgttcaagtacaaaatagtacaaaaacggagatagaaccaaacaatcgtccagaagaagccactatgcttccatttcatacaccactaagcggtagtttaatggaggatgatcatacggatgtatacgaattcaatgttacatctcctaaagaaatagatatatctgttttaaatgaaaaccaaattggcatgacatgggtgctttatcatgaatcagatagccaaaattatgcgtcttttggacaggaagacggaaacatgataaacggtaaattgaatgcaaagcctggaaagtattatttatatgtttataaatttgaaaatgagaacggaacatataccgttcatgtacagtaa

SEQ ID NO: 4 - DNA, 3219 bp, Lysinibacillus fusiformis
atgaagaaaaaatttacattcaatcagttgttaattggggttagtacaatggccatttcgttaggtggattacaggcggaagcatcggcagcagaaaaaacgccgtataatgtattacaaatgaaacccattggcatagaaatgtcgaaagatgaaatggtgcattcgacaatggctgaagaaacattatcctatgaagaacgtttagaaatgggagatttttcacaacgtccagcaccaattatggaacagatggatacacagcaattgcaggagcagtactcgatggcagagcttaataatatgagcaatcgtgagcttatccatacgcttggcagtatccgttggtaccaaattacagacttattccaattcaatgatgacacaaaagctttttatcaaaatgaagagcgcatgcaagtaatcatcaatgaattagggaatagaggaaattcgtttacgaaggaagattcaaaggggatcgaaacatttgttgaggtattgcgttctgctttttatgtagcgttttataataatgaactaggctatttaaatgagagaagtttccaagataagtgtttaccagcattaaatgaaatagccaaaaatccaaactttaaacttggtacagatgagcaagataaagttgtatctgcctatggaaaattaataggtaatgcttctagtgatgtggaaaccgttcaacatgctacgaacattttaaaacaatataatgaaaatctttctacctatgaaagtgagaattcaaaaggacaagctatttacgatataatacacggcattgattatgatttgcagtcttatttatatgacactcgtaaagaggccaatacaacgatgtggtatgggaagattgatagcttcatagaggaagttaataacattgccctaatacataatgtgacggatagcaatagttggttaattaataatggcatttattatgcagggcgtttagggcagttccatagcaatcctaataagggtttagaagtcgttacacaagcgatgcatatgtatccctatttaagtgaagcttattttgtggcagtagagcaaattacgacaaattatggtggacgtgacttaaacggaaatacggttgatttacaaaaagtacgtgaagaaggaaaaaaacagtatctaccgaaaacatatacatttgatgatggatcaattgtattcaaaacgggagatcaagtaacggaagataaaattcaaagattatactgggctgcaaaagaggtaaaggcacaatatcatcgtgtaatcgggaatgatcaagcactagagcctggtaatgctgacgatatcttaaccgttgtcatttataactctcccgatcagtaccgattaaaccgacaattgtacggatatgaaacaaataatggtggtatttatattgaagagactggaacattctttacatatgaacgtacacctgagcaaagtatttatagcttagaagagctgttccgtcatgaatatacgcactttttacaaggtagatttgaggtgcctggtctattcgggacgggtgatatgtatcaaaatgagcgactaacatggttccaggaagggaatgcagaattttttgcagggtcaacacgtacaaatgacgttgtgcctcgtaagagcattattagtggattgtcacaggatccatcacaacgctatactgctgaacaaacaatgtttgccacatatggttcctgggatttttataattattcatttgcattacagtcttatatgtatacgcatcaattcgatatgtttgatagaattcaagatttaatccgcgcgaacgatgtgaaaaattatgatgcctatcgtgacactttaagtaaagattcacagctgaatatggaataccaagcatatatgcagcaattgatcgataaccaagaaacatacgaagtaccacaagtagcagaggattatttaatgccgcatgaaccaaaagcgttaaacgaagtacagcaagaaattgtcgatattgcacatgtgaaagatgcaaatatgacgaaacaccagtctcaattttttaatacgtttacactcgagggaacatatgtaggtagtgcaacacagggtgaatctcaagattggaaaacgatgagtaagcaagtaaaccaaatgctggagcaactgtctcaaaaagagtggagcggctataaaacaatgactgcgtactttgtcaactatcgtgtaaatgcggcaaaccagttcgagtatgatgtagtcttccatggcgtttccactgatgacggagaaacgcaagcaccaattgtacaagtaaatggtccatatactggcatgatcaatgaaaaaattcaatttaatagtgatgggtcaaaggatacggatggagaaatagtttcttatctttgggattttggtgatggcgcgacaagtgaagcagcaaatcctactcatgtatacgaaaatgaaggaacttacaaagtgacgttaaccgtgaaaaataataagggacaagaaagtaaagggcaaacaactgccactgtacagaaaggaggacagacagggcaagaacatgcgatgattattccatttaataaaccactaaaaggtagtttgatagaaaatgatacaaatgtctatcaatttgacattacatcgccagaagaaatagatatttctgtcgtaaatgaaaatcaaattggcatgacatgggtgctttatcatgaatctgataaggaaaactatgtagcgtatggacaggaagatggacagacaataaaaggtaagtacaatgcgaaaccaggaaagtattatttatacgtttataagtttgatgatgaagatggaacatataccgttcaagtacaaaatagtacaaaaacggagatagaaccaaacaatcgtccagaagaagccactatgcttccatttcatacaccactaagcggtagtttaatggaggatgatcatacggatgtatacgaattcaatgttacatctcctaaagaaatagatatatctgttttaaatgaaaaccaaattggcatgacatgggtgctttatcatgaatcagatagccaaaattatgcgtcttttggacaggaagacggaaacatgataaacggtaaattgaatgcaaagcctggaaagtattatttatatgtttataaatttgaaaatgagaacggaacatataccgttcatgtacagtaa

SEQ ID NO: 5 - DNA, 21 bp, Artificial Sequence
  Forward primer
ggaaacaatctaaatgtgtct

SEQ ID NO: 6 - DNA, 21 bp, Artificial Sequence
  Reverse primer
ccgcctttaaaggctctccga